European Patent Application EP 4 328 236 A1, published February 28, 2024. Title: Glycosylated RBD and use thereof. Applicant: OSAKA UNIVERSITY. The sequence listing filed with the application follows.

SEQUENCE LISTING (114 sequences)

SEQ ID NO: 1 - protein, 1273 aa, SARS-CoV-2
MFVFLVLLPLVSSQCVNLTTRTQLPPAYTNSFTRGVYYPDKVFRSSVLHSTQDLFLPFFSNVTWFHAIHVSGTNGTKRFDNPVLPFNDGVYFASTEKSNIIRGWIFGTTLDSKTQSLLIVNNATNVVIKVCEFQFCNDPFLGVYYHKNNKSWMESEFRVYSSANNCTFEYVSQPFLMDLEGKQGNFKNLREFVFKNIDGYFKIYSKHTPINLVRDLPQGFSALEPLVDLPIGINITRFQTLLALHRSYLTPGDSSSGWTAGAAAYYVGYLQPRTFLLKYNENGTITDAVDCALDPLSETKCTLKSFTVEKGIYQTSNFRVQPTESIVRFPNITNLCPFGEVFNATRFASVYAWNRKRISNCVADYSVLYNSASFSTFKCYGVSPTKLNDLCFTNVYADSFVIRGDEVRQIAPGQTGKIADYNYKLPDDFTGCVIAWNSNNLDSKVGGNYNYLYRLFRKSNLKPFERDISTEIYQAGSTPCNGVEGFNCYFPLQSYGFQPTNGVGYQPYRVVVLSFELLHAPATVCGPKKSTNLVKNKCVNFNFNGLTGTGVLTESNKKFLPFQQFGRDIADTTDAVRDPQTLEILDITPCSFGGVSVITPGTNTSNQVAVLYQDVNCTEVPVAIHADQLTPTWRVYSTGSNVFQTRAGCLIGAEHVNNSYECDIPIGAGICASYQTQTNSPRRARSVASQSIIAYTMSLGAENSVAYSNNSIAIPTNFTISVTTEILPVSMTKTSVDCTMYICGDSTECSNLLLQYGSFCTQLNRALTGIAVEQDKNTQEVFAQVKQIYKTPPIKDFGGFNFSQILPDPSKPSKRSFIEDLLFNKVTLADAGFIKQYGDCLGDIAARDLICAQKFNGLTVLPPLLTDEMIAQYTSALLAGTITSGWTFGAGAALQIPFAMQMAYRFNGIGVTQNVLYENQKLIANQFNSAIGKIQDSLSSTASALGKLQDVVNQNAQALNTLVKQLSSNFGAISSVLNDILSRLDKVEAEVQIDRLITGRLQSLQTYVTQQLIRAAEIRASANLAATKMSECVLGQSKRVDFCGKGYHLMSFPQSAPHGVVFLHVTYVPAQEKNFTTAPAICHDGKAHFPREGVFVSNGTHWFVTQRNFYEPQIITTDNTFVSGNCDVVIGIVNNTVYDPLQPELDSFKEELDKYFKNHTSPDVDLGDISGINASVVNIQKEIDRLNEVAKNLNESLIDLQELGKYEQYIKWPWYIWLGFIAGLIAIVMVTIMLCCMTSCCSCLKGCCSCGSCCKFDEDDSEPVLKGVKLHYT

SEQ ID NO: 2 - protein, 199 aa, SARS-CoV-2
NITNLCPFGEVFNATRFASVYAWNRKRISNCVADYSVLYNSASFSTFKCYGVSPTKLNDLCFTNVYADSFVIRGDEVRQIAPGQTGKIADYNYKLPDDFTGCVIAWNSNNLDSKVGGNYNYLYRLFRKSNLKPFERDISTEIYQAGSTPCNGVEGFNCYFPLQSYGFQPTNGVGYQPYRVVVLSFELLHAPATVCGPKK

SEQ ID NO: 3 - protein, 11 aa, Mus musculus
VRDYGYGYFDV

SEQ ID NO: 4 - protein, 11 aa, Mus musculus
VRGYGYGYFDV

SEQ ID NO: 5 - protein, 11 aa, Mus musculus
VRDYGYGYFDD

SEQ ID NO: 6 - protein, 12 aa, Mus musculus
AIITTVLPWFAY

SEQ ID NO: 7 - protein, 12 aa, Mus musculus
AIMTTVLPWFAY

SEQ ID NO: 8 - protein, 12 aa, Mus musculus
AIITTVAPFFAY

SEQ ID NO: 9 - protein, 12 aa, Mus musculus
AIITTVAPYFAY

SEQ ID NO: 10 - protein, 12 aa, Mus musculus
ALITTVLPWFAF

SEQ ID NO: 11 - protein, 12 aa, Mus musculus
ALITTVLPWFTF

SEQ ID NO: 12 - protein, 11 aa, Mus musculus
TRESDYGFFDY

SEQ ID NO: 13 - protein, 11 aa, Mus musculus
ARESDYGFFDC

SEQ ID NO: 14 - protein, 11 aa, Mus musculus
VRESDYGYFAY

SEQ ID NO: 15 - protein, 11 aa, Mus musculus
ARESDYGFFDY

SEQ ID NO: 16 - protein, 18 aa, Mus musculus
ARHGGTYYYGISPYAMDY

SEQ ID NO: 17 - protein, 18 aa, Mus musculus
ARHSGTYYYGSSPYAMDY

SEQ ID NO: 18 - protein, 18 aa, Mus musculus
ARHSGTYYYGSSPYGMDY

SEQ ID NO: 19 - protein, 11 aa, Mus musculus
ARGWLGHYFDY

SEQ ID NO: 20 - protein, 9 aa, Mus musculus
QHHYGTPLT

SEQ ID NO: 21 - protein, 9 aa, Mus musculus
QHHYGNPLT

SEQ ID NO: 22 - protein, 9 aa, Mus musculus
QHHYGSPLT

SEQ ID NO: 23 - protein, 9 aa, Mus musculus
QHHYDAPLT

SEQ ID NO: 24 - protein, 9 aa, Mus musculus
QHHYGAPLT

SEQ ID NO: 25 - protein, 8 aa, Mus musculus
HQYLSSWT

SEQ ID NO: 26 - protein, 10 aa, Mus musculus
QHHYGSPPWT

SEQ ID NO: 27 - protein, 10 aa, Mus musculus
QHHYGTPPWT

SEQ ID NO: 28 - protein, 9 aa, Mus musculus
QHFWDTPYT

SEQ ID NO: 29 - protein, 9 aa, Mus musculus
QQHYSTPRT

SEQ ID NO: 30 - protein, 11 aa, Mus musculus
TIGYGYGYFDY

SEQ ID NO: 31 - protein, 11 aa, Mus musculus
TKGYGYGYFDY

SEQ ID NO: 32 - protein, 11 aa, Mus musculus
TKGYGYGYFDQ

SEQ ID NO: 33 - protein, 11 aa, Mus musculus
SIGYGYGYFDY

SEQ ID NO: 34 - protein, 6 aa, Mus musculus
ARNFDV

SEQ ID NO: 35 - protein, 6 aa, Mus musculus
ARYFDV

SEQ ID NO: 36 - protein, 11 aa, Mus musculus
VRDYGYGYFGV

SEQ ID NO: 37 - protein, 11 aa, Mus musculus
TIGFGYGYFDY

SEQ ID NO: 38 - protein, 12 aa, Mus musculus
ARHYDYDDGMDY

SEQ ID NO: 39 - protein, 11 aa, Mus musculus
ARYGNDWYFDV

SEQ ID NO: 40 - protein, 15 aa, Mus musculus
TTPVYDGYYDYAMDC

SEQ ID NO: 41 - protein, 9 aa, Mus musculus
QHHYGTPYT

SEQ ID NO: 42 - protein, 9 aa, Mus musculus
QHHYGSPYT

SEQ ID NO: 43 - protein, 9 aa, Mus musculus
QQWNNYPYT

SEQ ID NO: 44 - protein, 9 aa, Mus musculus
QQWSSYPYT

SEQ ID NO: 45 - protein, 9 aa, Mus musculus
QHHYGPPYT

SEQ ID NO: 46 - protein, 9 aa, Mus musculus
QHHYGPPFT

SEQ ID NO: 47 - protein, 9 aa, Mus musculus
  misc_feature (9)..(9): Xaa can be any naturally occurring amino acid
FQGSHVPRX

SEQ ID NO: 48 - protein, 9 aa, Mus musculus
QQGGEDPWT

SEQ ID NO: 49 - protein, 15 aa, Mus musculus
ARLDSSYYVDYPMDY

SEQ ID NO: 50 - protein, 15 aa, Mus musculus
ARLDSSYYVDYPLDY

SEQ ID NO: 51 - protein, 15 aa, Mus musculus
ARLDSSAYVDYPMDY

SEQ ID NO: 52 - protein, 15 aa, Mus musculus
VRLDSSAYVGYPMDY

SEQ ID NO: 53 - protein, 15 aa, Mus musculus
ARLDTSSYVDYAMDY

SEQ ID NO: 54 - protein, 15 aa, Mus musculus
ARLDSSAYVEYPMDY

SEQ ID NO: 55 - protein, 15 aa, Mus musculus
ARLDSSTYVDYAMDY

SEQ ID NO: 56 - protein, 15 aa, Mus musculus
ARLDSSAYVGYAMDY

SEQ ID NO: 57 - protein, 15 aa, Mus musculus
ARLDSSAYVDYPMDF

SEQ ID NO: 58 - protein, 15 aa, Mus musculus
ARLDSSAYLGYPLDY

SEQ ID NO: 59 - protein, 15 aa, Mus musculus
ARLDSSGYVGYAMDY

SEQ ID NO: 60 - protein, 15 aa, Mus musculus
ARLDSAAYVGYAMDY

SEQ ID NO: 61 - protein, 15 aa, Mus musculus
IRLDSSYYVDYPVDY

SEQ ID NO: 62 - protein, 15 aa, Mus musculus
ARLDSSYYVDYPVDY

SEQ ID NO: 63 - protein, 15 aa, Mus musculus
ARLDISDYVDYPMDH

SEQ ID NO: 64 - protein, 15 aa, Mus musculus
ARLDSSSYVDYPMDY

SEQ ID NO: 65 - protein, 15 aa, Mus musculus
ARLDSSAYVGYPMDY

SEQ ID NO: 66 - protein, 15 aa, Mus musculus
ARLDSSCYVDYPVDY

SEQ ID NO: 67 - protein, 15 aa, Mus musculus
ARLDSSYFVDYPLDS

SEQ ID NO: 68 - protein, 15 aa, Mus musculus
VRLDSSYYVDYPVDY

SEQ ID NO: 69 - protein, 17 aa, Mus musculus
ARQRGSYYRYDDYAMDY

SEQ ID NO: 70 - protein, 14 aa, Mus musculus
ARWGNYVSYYTMDY

SEQ ID NO: 71 - protein, 9 aa, Mus musculus
LQYDEFPYT

SEQ ID NO: 72 - protein, 9 aa, Mus musculus
LQYDEFPFT

SEQ ID NO: 73 - protein, 9 aa, Mus musculus
QQYDEFPYT

SEQ ID NO: 74 - protein, 9 aa, Mus musculus
LQYDDFPYT

SEQ ID NO: 75 - protein, 9 aa, Mus musculus
LQYAEFPYT

SEQ ID NO: 76 - protein, 9 aa, Mus musculus
LHYDEFPYT

SEQ ID NO: 77 - protein, 9 aa, Mus musculus
FQGSHVPWT

SEQ ID NO: 78 - protein, 11 aa, Mus musculus
QHYHSYPPMWT

SEQ ID NO: 79 - protein, 15 aa, Mus musculus
ARLDYDGYYEYAMDY

SEQ ID NO: 80 - protein, 15 aa, Mus musculus
ARLDYDTYYEYAMDY

SEQ ID NO: 81 - protein, 15 aa, Mus musculus
ARLDFDGYYEYPMDY

SEQ ID NO: 82 - protein, 15 aa, Mus musculus
SRLDFDGYYEYAMDY

SEQ ID NO: 83 - protein, 15 aa, Mus musculus
TRLDYDGYYDYAVDY

SEQ ID NO: 84 - protein, 15 aa, Mus musculus
TRLDYDGYYDYAMDY

SEQ ID NO: 85 - protein, 15 aa, Mus musculus
ARLDYDGYYDFAMDY

SEQ ID NO: 86 - protein, 15 aa, Mus musculus
ARLDYDGYYEYPMDY

SEQ ID NO: 87 - protein, 15 aa, Mus musculus
ARLDYDGYYENAMDY

SEQ ID NO: 88 - protein, 15 aa, Mus musculus
ARLDYDAYYEYAMDY

SEQ ID NO: 89 - protein, 15 aa, Mus musculus
ARLDYAGYYEYAMDY

SEQ ID NO: 90 - protein, 15 aa, Mus musculus
TRLDYEGYYEYAMDY

SEQ ID NO: 91 - protein, 15 aa, Mus musculus
TRLDYDSYYEYALDY

SEQ ID NO: 92 - protein, 15 aa, Mus musculus
SRLDYDGYYEYAMDY

SEQ ID NO: 93 - protein, 15 aa, Mus musculus
SRLDYDGYYEYTMDY

SEQ ID NO: 94 - protein, 15 aa, Mus musculus
ARLDYDGYYDYALDY

SEQ ID NO: 95 - protein, 15 aa, Mus musculus
ARLDYDGYYEYPLDY

SEQ ID NO: 96 - protein, 15 aa, Mus musculus
ARLDYDGYYDYAMDY

SEQ ID NO: 97 - protein, 15 aa, Mus musculus
ARLDYDGYYEYAVDY

SEQ ID NO: 98 - protein, 15 aa, Mus musculus
ARLDYDGYYEYALDY

SEQ ID NO: 99 - protein, 15 aa, Mus musculus
ARLDYDAYYENAMDY

SEQ ID NO: 100 - protein, 15 aa, Mus musculus
GRLDSLHYYDYGFDY

SEQ ID NO: 101 - protein, 15 aa, Mus musculus
VRLDYDGYYEYSMDY

SEQ ID NO: 102 - protein, 15 aa, Mus musculus
TRLDYDGYYEYALDY

SEQ ID NO: 103 - protein, 12 aa, Mus musculus
ARDGGDYDWFAY

SEQ ID NO: 104 - protein, 9 aa, Mus musculus
LQYDEFPRT

SEQ ID NO: 105 - protein, 9 aa, Mus musculus
LQYDDFPRT

SEQ ID NO: 106 - protein, 8 aa, Mus musculus
QHHYGSST

SEQ ID NO: 107 - protein, 199 aa, Pangolin-GX-P2V
NITNLCPFGEVFNASKFASVYAWNRKRISNCVADYSVLYNSTSFSTFKCYGVSPTKLNDLCFTNVYADSFVVKGDEVRQIAPGQTGVIADYNYKLPDDFTGCVIAWNSVKQDALTGGNYGYLYRLFRKSKLKPFERDISTEIYQAGSTPCNGQVGLNCYYPLERYGFHPTTGVNYQPFRVVVLSFELLNGPATVCGPKL

SEQ ID NO: 108 - protein, 198 aa, SARS-CoV-1
NITNLCPFGEVFNATKFPSVYAWERKKISNCVADYSVLYNSTFFSTFKCYGVSATKLNDLCFSNVYADSFVVKGDDVRQIAPGQTGVIADYNYKLPDDFMGCVLAWNTRNIDATSTGNYNYKYRYLRHGKLRPFERDISNVPFSPDGKPCTPPALNCYWPLNDYGFYTTTGIGYQPYRVVVLSFELLNAPATVCGPKL

SEQ ID NO: 109 - protein, 198 aa, WIV1
NITNLCPFGEVFNATTFPSVYAWERKRISNCVADYSVLYNSTSFSTFKCYGVSATKLNDLCFSNVYADSFVVKGDDVRQIAPGQTGVIADYNYKLPDDFTGCVLAWNTRNIDATQTGNYNYKYRSLRHGKLRPFERDISNVPFSPDGKPCTPPAFNCYWPLNDYGFYITNGIGYQPYRVVVLSFELLNAPATVCGPKL

SEQ ID NO: 110 - protein, 198 aa, SHC014
NITNLCPFGEVFNATTFPSVYAWERKRISNCVADYSVLYNSTSFSTFKCYGVSATKLNDLCFSNVYADSFVVKGDDVRQIAPGQTGVIADYNYKLPDDFLGCVLAWNTNSKDSSTSGNYNYLYRWVRRSKLNPYERDLSNDIYSPGGQSCSAVGPNCYNPLRPYGFFTTAGVGHQPYRVVVLSFELLNAPATVCGPKL

SEQ ID NO: 111 - protein, 180 aa, Anlong-103
NITNRCPFDSIFNASRFPSVYAWERTKISDCVADYTVLYNSTSFSTFKCYGVSPSKLIDLCFTSVYADTFLIRFSEVRQVAPGETGVIADYNYRLPDDFTGCVIAWNTANQDVGSYFYRSHRSTKLKPFERDLSSDENGVRTLSTYDFNPYVPLDYQATRVVVLSFELLNAPATVCGPKL

SEQ ID NO: 112 - protein, 180 aa, Rf1-2004
NITNLCPFDKVFNATRFPSVYAWERTKISDCVADYTVFYNSTSFSTFNCYGVSPSKLIDLCFTSVYADTFLIRFSEVRQVAPGQTGVIADYNYKLPDDFTGCVIAWNTAKQDVGSYFYRSHRSSKLKPFERDLSSEENGVRTLSTYDFNQNVPLEYQATRVVVLSFELLNAPATVCGPKL

SEQ ID NO: 113 - protein, 180 aa, Rs4081
NITNRCPFDKVFNASRFPNVYAWERTKISDCVADYTVLYNSTSFSTFKCYGVSPSKLIDLCFTSVYADTFLIRSSEVRQVAPGETGVIADYNYKLPDDFTGCVIAWNTAKQDQGQYYYRSSRKTKLKPFERDLTSDENGVRTLSTYDFYPNVPIEYQATRVVVLSFELLNAPATVCGPKL

SEQ ID NO: 114 - protein, 195 aa, BM48-31
NITQLCPFNEVFNITSFPSVYAWERMRITNCVADYSVLYNSSASFSTFQCYGVSPTKLNDLCFSSVYADYFVVKGDDVRQIAPAQTGVIADYNYKLPDDFTGCVIAWNTNSLDSSNEFFYRRFRHGKIKPYGRDLSNVLFNPSGGTCSAEGLNCYKPLASYGFTQSSGIGFQPYRVVVLSFELLNAPATVCGPKQ